European Patent Specification EP 3 584 322 B1, published December 4, 2024. Title: CONSTITUTIVE PROMOTER. Applicant: Lonza Ltd. The sequence listing filed with the application follows.

SEQUENCE LISTING (24 sequences)

SEQ ID NO: 1 - DNA, 985 bp, Pichia pastoris
agggcatcattgaggtttccacaaaaggaagaaacatggatccagagacatcaacagagaggaaagcgggtagtgaagccgaagccacaacacagcccgatttggaagggagttcacaatcaaggtgagtccagccattttttttcttttttttttttttattcaggtgaacccacctaactatttttaactgggatccagtgagctcgctgggtgaaagccaaccatcttttgtttcggggaaccgtgctcgccccgtaaagttaatttttttttcccgcgcagctttaatctttcggcagagaaggcgttttcatcgtagcgtgggaacagaataatcagttcatgtgctatacaggcacatggcagcagtcactattttgctttttaaccttaaagtcgttcatcaatcattaactgaccaatcagattttttgcatttgccacttatctaaaaatacttttgtatctcgcagatacgttcagtggtttccaggacaacacccaaaaaaaggtatcaatgccactaggcagtcggttttatttttggtcacccacgcaaagaagcacccacctcttttaggttttaagttgtgggaacagtaacaccgcctagagcttcaggaaaaaccagtacctgtgaccgcaattcaccatgatgcagaatgttaatttaaacgagtgccaaatcaagatttcaacagacaaatcaatcgatccatagttacccattccagccttttcgtcgtcgagcctgcttcattcctgcctcaggtgcataactttgcatgaaaagtccagattagggcagattttgagtttaaaataggaaatataaacaaatataccgcgaaaaaggtttgtttatagcttttcgcctggtgccgtacggtataaatacatactctcctcccccccctggttctctttttcttttgttacttacattttaccgttccgtcactcgcttcactcaacaacaaaa

SEQ ID NO: 2 - DNA, 1488 bp, Pichia pastoris
gatagttctagaagacctggcgtcgctggtcaactactcgtttcacaagttgacaaagacttttaccaagagaagagcagttgtcaccgaccacaataacaacctggaagccgagaaaaaacttggaatctccaaggtgagactgcctagaaatccgtactctgcggccgatcgaagactgcatttcctccaagaattgatgctcatggtctcatcttacaatcgcacacacaacagtgtcagtcttctttgcggtcccttgaacacaaccaaccgaaaggtggggaagtctaatgtcacgcaaacgatattgcaaccaatgttgggctctactggcgtctggctgcatcaaatagctgatcggttcgtaatcttcaaagattggtgtaggacgaacgagtctgctgggctacaagttttgccccatatcgctgttcaagccaacccgcggaatcccaaaacaccccatccgacaaaagttgttgttttcagcagatctagggagggcatcattgaggtttccacaaaaggaagaaacatggatccagagacatcaacagagaggaaagcgggtagtgaagccgaagccacaacacagcccgatttggaagggagttcacaatcaaggtgagtccagccattttttttcttttttttttttttattcaggtgaacccacctaactatttttaactgggatccagtgagctcgctgggtgaaagccaaccatcttttgtttcggggaaccgtgctcgccccgtaaagttaatttttttttcccgcgcagctttaatctttcggcagagaaggcgttttcatcgtagcgtgggaacagaataatcagttcatgtgctatacaggcacatggcagcagtcactattttgctttttaaccttaaagtcgttcatcaatcattaactgaccaatcagattttttgcatttgccacttatctaaaaatacttttgtatctcgcagatacgttcagtggtttccaggacaacacccaaaaaaaggtatcaatgccactaggcagtcggttttatttttggtcacccacgcaaagaagcacccacctcttttaggttttaagttgtgggaacagtaacaccgcctagagcttcaggaaaaaccagtacctgtgaccgcaattcaccatgatgcagaatgttaatttaaacgagtgccaaatcaagatttcaacagacaaatcaatcgatccatagttacccattccagccttttcgtcgtcgagcctgcttcattcctgcctcaggtgcataactttgcatgaaaagtccagattagggcagattttgagtttaaaataggaaatataaacaaatataccgcgaaaaaggtttgtttatagcttttcgcctggtgccgtacggtataaatacatactctcctcccccccctggttctctttttcttttgttacttacattttaccgttccgtcactcgcttcactcaacaacaaaa

SEQ ID NO: 3 - DNA, 767 bp, Pichia pastoris
agccaaccatcttttgtttcggggaaccgtgctcgccccgtaaagttaatttttttttcccgcgcagctttaatctttcggcagagaaggcgttttcatcgtagcgtgggaacagaataatcagttcatgtgctatacaggcacatggcagcagtcactattttgctttttaaccttaaagtcgttcatcaatcattaactgaccaatcagattttttgcatttgccacttatctaaaaatacttttgtatctcgcagatacgttcagtggtttccaggacaacacccaaaaaaaggtatcaatgccactaggcagtcggttttatttttggtcacccacgcaaagaagcacccacctcttttaggttttaagttgtgggaacagtaacaccgcctagagcttcaggaaaaaccagtacctgtgaccgcaattcaccatgatgcagaatgttaatttaaacgagtgccaaatcaagatttcaacagacaaatcaatcgatccatagttacccattccagccttttcgtcgtcgagcctgcttcattcctgcctcaggtgcataactttgcatgaaaagtccagattagggcagattttgagtttaaaataggaaatataaacaaatataccgcgaaaaaggtttgtttatagcttttcgcctggtgccgtacggtataaatacatactctcctcccccccctggttctctttttcttttgttacttacattttaccgttccgtcactcgcttcactcaacaacaaaa

SEQ ID NO: 4 - DNA, 500 bp, Pichia pastoris
gtggtttccaggacaacacccaaaaaaaggtatcaatgccactaggcagtcggttttatttttggtcacccacgcaaagaagcacccacctcttttaggttttaagttgtgggaacagtaacaccgcctagagcttcaggaaaaaccagtacctgtgaccgcaattcaccatgatgcagaatgttaatttaaacgagtgccaaatcaagatttcaacagacaaatcaatcgatccatagttacccattccagccttttcgtcgtcgagcctgcttcattcctgcctcaggtgcataactttgcatgaaaagtccagattagggcagattttgagtttaaaataggaaatataaacaaatataccgcgaaaaaggtttgtttatagcttttcgcctggtgccgtacggtataaatacatactctcctcccccccctggttctctttttcttttgttacttacattttaccgttccgtcactcgcttcactcaacaacaaaa

SEQ ID NO: 5 - DNA, 344 bp, Pichia pastoris
gaccgcaattcaccatgatgcagaatgttaatttaaacgagtgccaaatcaagatttcaacagacaaatcaatcgatccatagttacccattccagccttttcgtcgtcgagcctgcttcattcctgcctcaggtgcataactttgcatgaaaagtccagattagggcagattttgagtttaaaataggaaatataaacaaatataccgcgaaaaaggtttgtttatagcttttcgcctggtgccgtacggtataaatacatactctcctcccccccctggttctctttttcttttgttacttacattttaccgttccgtcactcgcttcactcaacaacaaaa

SEQ ID NO: 6 - DNA, 234 bp, Pichia pastoris
agcctgcttcattcctgcctcaggtgcataactttgcatgaaaagtccagattagggcagattttgagtttaaaataggaaatataaacaaatataccgcgaaaaaggtttgtttatagcttttcgcctggtgccgtacggtataaatacatactctcctcccccccctggttctctttttcttttgttacttacattttaccgttccgtcactcgcttcactcaacaacaaaa

SEQ ID NO: 7 - DNA, 138 bp, Pichia pastoris
ccgcgaaaaaggtttgtttatagcttttcgcctggtgccgtacggtataaatacatactctcctcccccccctggttctctttttcttttgttacttacattttaccgttccgtcactcgcttcactcaacaacaaaa

SEQ ID NO: 8 - DNA, 85 bp, Pichia pastoris
catactctcctcccccccctggttctctttttcttttgttacttacattttaccgttccgtcactcgcttcactcaacaacaaaa

SEQ ID NO: 9 - DNA, 408 bp, Pichia pastoris
atgcaattctctatcgtcgctactttggctcttgctggttccgctctggctgcttactctaacgtaacttacacttacgagactaccatcaccgatgttgtcaccgagctcaccacttactgcccagagccaaccaccttcgttcacaagaacaagaccatcactgtgaccgccccaaccactttgaccatcactgactgtccttgcaccatctccaagaccaccaagatcaccactgatgttccaccaaccacccactccaccccacacaccaccaccactcacgtgccatctacctctaccccagctccaacccactctgtttctaccatctctcacggtggtgctgctaaggctggtgttgctggtttggccggtgttgctgctgccgctgcttacttcttgtaa

SEQ ID NO: 10 - protein, 135 aa, Pichia pastoris
MQFSIVATLALAGSALAAYSNVTYTYETTITDVVTELTTYCPEPTTFVHKNKTITVTAPTTLTITDCPCTISKTTKITTDVPPTTHSTPHTTTTHVPSTSTPAPTHSVSTISHGGAAKAGVAGLAGVAAAAAYFL

SEQ ID NO: 11 - DNA, 402 bp, Pichia pastoris
atgcaattctctatcgtcgctactttggctcttgctggttccgctctggctgcttactctaacgtaacttacacttacgagactaccatcaccgatgttgtcactgagttgaccacttactgcccagagccaaccacctttgtttacaagaacaagaccatcaccgtgactgagccaaccactttgaccatcactgactgcccatgcaccatctcaaagaccaccaagatcaccactgatgttccaccaaccacccacgtcaccccatccaccactcacgtgccatctacctctaccccagctccaacccactctgtttctaccatctctcacggtggtgctgctaaggctggtgttgctggtttggccggtgttgctgctgccgctgcttacttcttgtaa

SEQ ID NO: 12 - protein, 133 aa, Pichia pastoris
MQFSIVATLALAGSALAAYSNVTYTYETTITDVVTELTTYCPEPTTFVYKNKTITVTEPTTLTITDCPCTISKTTKITTDVPPTTHVTPSTTHVPSTSTPAPTHSVSTISHGGAAKAGVAGLAGVAAAAAYFL

SEQ ID NO: 13 - DNA, 491 bp, Pichia pastoris
cttttttgtagaaatgtcttggtgtcctcgtccaatcaggtagccatctctgaaatatctggctccgttgcaactccgaacgacctgctggcaacgtaaaattctccggggtaaaacttaaatgtggagtaatggaaccagaaacgtctcttcccttctctctccttccaccgcccgttaccgtccctaggaaattttactctgctggagagcttcttctacggcccccttgcagcaatgctcttcccagcattacgttgcgggtaaaacggaggtcgtgtacccgacctagcagcccagggatggaaaagtcccggccgtcgctggcaataatagcgggcggacgcatgtcatgagattattggaaaccaccagaatcgaatataaaaggcgaacacctttcccaattttggtttctcctgacccaaagactttaaatttaatttatttgtccctatttcaatcaattgaacaactatcacctgcaggcc

SEQ ID NO: 14 - DNA, 33 bp, artificial
  Primer
gatagggccccagggcatcattgaggtttccac

SEQ ID NO: 15 - DNA, 36 bp, artificial
  Primer
gatacctgcaggttttgttgttgagtgaagcgagtg

SEQ ID NO: 16 - DNA, 33 bp, artificial; identical to SEQ ID NO: 14
  Primer

SEQ ID NO: 17 - DNA, 35 bp, artificial
  Primer
gatagggcccgatagttctagaagacctggcgtcg

SEQ ID NO: 18 - DNA, 31 bp, artificial
  Primer
gatagggcccagccaaccatcttttgtttcg

SEQ ID NO: 19 - DNA, 31 bp, artificial
  Primer
gatagggcccgtggtttccaggacaacaccc

SEQ ID NO: 20 - DNA, 31 bp, artificial
  Primer
gatagggcccgaccgcaattcaccatgatgc

SEQ ID NO: 21 - DNA, 29 bp, artificial
  Primer
gatagggcccagcctgcttcattcctgcc

SEQ ID NO: 22 - DNA, 33 bp, artificial
  Primer
gatagggcccccgcgaaaaaggtttgtttatag

SEQ ID NO: 23 - DNA, 31 bp, artificial
  Primer
gatagggccccatactctcctcccccccctg

SEQ ID NO: 24 - DNA, 345 bp, artificial
  translational fusion partner
ggccattacggccgggggacttacattttaccgttccgtcactcgcttcactcaacaacaaaaatgcaattctctatcgtcgctactttggctcttgctggttccgctctggctgcttactctaacgtaacttacacttacgagactaccatcaccgatgttgtcaccgagctcaccacttactgcccagagccaaccaccttcgttcacaagaacaagaccatcactgtgaccgccccaaccactttgaccatcactgactgtccttgcaccatctccaagaccaccaagatcaccactgatgttccaccaaccacccactccaccccactggccgcctcggcc